European Patent Specification EP 3 486 311 B1, published November 15, 2023. Title: Leuconostoc mesenteroides CJLM181 producing decreased amounts of gas and methods for preparing kimchi using the same. Applicant: CJ Cheiljedang Corporation. The sequence listing filed with the application follows.

SEQUENCE LISTING (2 sequences)

SEQ ID NO: 1 - RNA, 986 nt, Unknown
  16s rRNA sequences of Leuconostoc mesenteroides CJLM181
aaaagttcgggtctccagcggacacttaatgcgttagcttcggcactaagaggcggaaacctcctaacacctagtgttcatcgtttacggtgtggactaccagggtatctaatcctgtttgctacccacactttcgagcctcaacgtcagttgcagtccagtaagccgccttcgccactggtgttcttccatatatctacgcattccaccgctacacatggagttccacttacctctactgcactcaagttaaccagtttccaatgccattccggagttgagctccgggctttcacatcagacttaataaaccgtctgcgctcgctttacgcccaataaatccggataacgctcgggacatacgtattaccgcggctgctggcacgtatttagccgtccctttctggtatggtaccgtcaaactaaaatcatttcctattctagctgttcttcccatacaacagtgctttacgacccgaaagccttcatcacacacgcggcgttgctccatcaggctttcgcccattgtggaagattccctactgcagcctcccgtaggagtttgggccgtgtctcagtcccaatgtggccgatcagtctctcaactcggctatgcatcattgtcttggtaggcctttaccccaccaactaactaatgcaccgcggatccatctctaggtgacgccgaagcgccttttaactttttgtcatgcgacactaagttttattcggtattagcatctgtttccaaatgttatccccagccttgaggcaggttgtccacgtgttactcacccgttcgccactcacttgaaaggtgcaagcacctttcgctgtgcgttcgacttgcatgtattaggcacgccgccagcgttcatcctgacagagaaaaaaaaactatataaagggttttggggtaaaatttttaaggaatttagggaccaaaggtaaaaagcttaaaagggttccctggttaccgatgtttg

SEQ ID NO: 2 - RNA, 1514 nt, Unknown
  16s rRNA sequences of Leuconostoc mesenteroides subsp. mesenteroides strain CCMMB1121
gctcaggatgaacgctggcggcgtgcctaatacatgcaagtcgaacgcacagcgaaaggtgcttgcacctttcaagtgagtggcgaacgggtgagtaacacgtggacaacctgcctcaaggctggggataacatttggaaacagatgctaataccgaataaaacttagtgtcgcatgacaaaaagttaaaaggcgcttcggcgtcacctagagatggatccgcggtgcattagttagttggtggggtaaaggcctaccaagacaatgatgcatagccgagttgagagactgatcggccacattgggactgagacacggcccaaactcctacgggaggctgcagtagggaatcttccacaatgggcgaaagcctgatggagcaacgccgcgtgtgtgatgaaggctttcgggtcgtaaagcactgttgtatgggaagaacagctagaataggaaatgattttagtttgacggtaccataccagaaagggacggctaaatacgtgccagcagccgcggtaatacgtatgtcccgagcgttatccggatttattgggcgtaaagcgagcgcagacggtttattaagtctgatgtgaaagcccggagctcaactccggaatggcattggaaactggttaacttgagtgcagtagaggtaagtggaactccatgtgtagcggtggaatgcgtagatatatggaagaacaccagtggcgaaggcggcttactggactgcaactgacgttgaggctcgaaagtgtgggtagcaaacaggattagataccctggtagtccacaccgtaaacgatgaacactaggtgttaggaggtttccgcctcttagtgccgaagctaacgcattaagtgttccgcctggggagtacgaccgcaaggttgaaactcaaaggaattgacggggacccgcacaagcggtggagcatgtggtttaattcgaagcaacgcgaagaaccttaccaggtcttgacatcctttgaagcttttagagatagaagtgttctcttcggagacaaagtgacaggtggtgcatggtcgtcgtcagctcgtgtcgtgagatgttgggttaagtcccgcaacgagcgcaacccttattgttagttgccagcattcagatgggcactctagcgagactgccggtgacaaaccggaggaaggcggggacgacgtcagatcatcatgccccttatgacctgggctacacacgtgctacaatggcgtatacaacgagttgccaacccgcgagggtgagctaatctcttaaagtacgtctcagttcggattgtagtctgcaactcgactacatgaagtcggaatcgctagtaatcgcggatcagcacgccgcggtgaatacgttcccgggtcttgtacacaccgcccgtcacaccatgggagtttgtaatgcccaaagccggtggcctaaccttttaggaaggagccgtctaaggcaggacagatgactggggtgaagtcgtaacaaggtagccgtaggagaacctgcgg